European Patent Application EP 4 303 231 A1, published January 10, 2024. Title: BISPECIFIC ANTIBODY. Applicant: CHIA TAI TIANQING PHARMACEUTICAL GROUP CO., LTD. The sequence listing filed with the application follows.

SEQUENCE LISTING (53 sequences)

SEQ ID NO: 1 - protein, 103 aa, Artificial Sequence
  Amino acid sequence of MHCICαori
GKETLQRADPPKTHVTHHPISDHEATLRCWALGFYPAEITLTWQRDGEDQTQDTELVETRPAGDRTFQKWAAVVVPSGEEQRYTCHVQHEGLPKPLTLRWEPS

SEQ ID NO: 2 - protein, 97 aa, Artificial Sequence
  Amino acid sequence of MHCICβori
IQRTPKIQVYSRHPAENGKSNFLNCYVSGFHPSDIEVDLLKNGERIEKVEHSDLSFSKDWSFYLLYYTEFTPTEKDEYACRVNHVTLSQPKIVKWDR

SEQ ID NO: 3 - protein, 103 aa, Artificial Sequence
  Optimized amino acid sequence of Cα
GKETLQRADPPKTHVTHHPISRHEATLRCWALGFYPAEITLTWQRDGKDQTQKTELVETRPCGDRTFQKWAAVVVPSGEEQRYTCHVQHEGLPKPLTLRWEPS

SEQ ID NO: 4 - protein, 99 aa, Artificial Sequence
  Optimized amino acid sequence of Cβ
IQRTPKIQVYSCHPAENGKSNFLNCYVSGFHPSDIEVDLLKNGERIEKVEHSDLSFSKDWSFYLLYYTRFTPTEKDEYACRVNHVTLSQPKIVKWDRGP

SEQ ID NO: 5 - protein, 97 aa, Artificial Sequence
  Amino acid sequence of another embodiment of Cβ
IQRTPKIQVYSCHPAENGKSNFLNCYVSGFHPSDIEVDLLKNGERIEKVEHSDLSFSKDWSFYLLYYTRFTPTEKDEYACRVNHVTLSQPKIVKWDR

SEQ ID NO: 6 - protein, 448 aa, Artificial Sequence
  Amino acid sequence of polypeptide chain H1 of MHI383-1122-IgG4
EVQLLESGGGLVQPGGSLRLSCAVSGFTFNSFAMSWVRQAPGKGLEWVSAISGSGGGTYYADSVKGRFTISRDNSKNTLYLQMNSLRAEDTAVYFCAKDKILWFGEPVFDYWGQGTLVTVSSASTKGPSVFPLAPCSRSTSESTAALGCLVKDYFPEPVTVSWNSGALTSGVHTFPAVLQSSGLYSLSSVVTVPSSSLGTKTYTCNVDHKPSNTKVDKRVESKYGPPCPPCPAPEFLGGPSVFLFPPKPKDTLMISRTPEVTCVVVDVSQEDPEVQFNWYVDGVEVHNAKTKPREEQFNSTYRVVSVLTVLHQDWLNGKEYKCKVSNKGLPSSIEKTISKAKGQPREPQVYTLPPCQEEMTKNQVSLWCLVKGFYPSDIAVEWESNGQPENNYKTTPPVLDSDGSFFLYSRLTVDKSRWQEGNVFSCSVMHEALHNHYTQKSLSLSLG

SEQ ID NO: 7 - DNA, 1344 bp, Artificial Sequence
  Nucleotide sequence of polypeptide chain H1 of MHI383-1122-IgG4
gaggtgcagctgctggagagcggaggaggactggtgcagccaggaggcagcctgagactgtcttgcgccgtgtccggcttcacctttaacagcttcgccatgtcttgggtgcgccaggctcctggcaagggactggagtgggtgtctgccatctctggatccggaggaggaacatactatgctgactccgtgaagggcaggttcaccatctcccgggataacagcaagaatacactgtacctgcagatgaattctctgagggccgaggacaccgccgtgtacttttgtgctaaggataagatcctgtggttcggcgagccagtgtttgactactggggccagggcaccctggtgacagtgtccagcgcctctacaaagggcccttccgtgttcccactggctccttgctctcgctccacaagcgagtctaccgccgctctgggctgtctggtgaaggactacttccccgagcctgtgaccgtgtcttggaattccggcgccctgacaagcggagtgcacacctttcctgctgtgctgcagtcttccggcctgtactctctgagctctgtggtgacagtgccttccagctctctgggcaccaagacatatacctgcaacgtggaccataagccatctaataccaaggtggataagagagtggagagcaagtacggaccaccatgccctccatgtcctgctccagagttcctgggaggaccatccgtgttcctgtttccacctaagcctaaggacacactgatgatcagccggacaccagaggtgacctgcgtggtggtggacgtgtctcaggaggatcccgaggtgcagttcaactggtacgtggatggcgtggaggtgcacaatgctaagaccaagcctagagaggagcagtttaattccacataccgcgtggtgagcgtgctgaccgtgctgcatcaggactggctgaacggcaaggagtataagtgtaaggtgtccaataagggcctgccatccagcatcgagaagaccatcagcaaggccaagggccagccaagagagccccaggtgtacacactgccaccctgccaggaggagatgaccaagaaccaggtgtccctgtggtgtctggtgaagggcttctatcccagcgacatcgctgtggagtgggagtctaatggccagcctgagaacaattacaagaccacacctccagtgctggacagcgatggctctttctttctgtattctaggctgacagtggataagtcccggtggcaggagggcaacgtgttttcttgctccgtgatgcacgaggccctgcacaatcattacacccagaagagcctgtctctgtccctgggc

SEQ ID NO: 8 - protein, 214 aa, Artificial Sequence
  Amino acid sequence of polypeptide chain L1 of MHI383-1122-IgG4
EIVLTQSPATLSLSPGERATLSCRASQSVSSYLAWYQQKPGQAPRLLIYDASNRATGIPARFSGSGSGTDFTLTISSLEPEDFAVYYCQQRSNWPPTFGQGTKVEIKRTVAAPSVFIFPPSDEQLKSGTASVVCLLNNFYPREAKVQWKVDNALQSGNSQESVTEQDSKDSTYSLSSTLTLSKADYEKHKVYACEVTHQGLSSPVTKSFNRGEC

SEQ ID NO: 9 - DNA, 642 bp, Artificial Sequence
  Nucleotide sequence of polypeptide chain L1 of MHI383-1122-IgG4
gagatcgtgctgacccagtctcctgccacactgagcctgtctccaggagagagggccaccctgtcctgcagggcttcccagagcgtgtccagctacctggcctggtatcagcagaagccaggccaggctcccaggctgctgatctacgacgccagcaacagagctaccggcatccccgctcgcttctctggatccggaagcggcacagactttaccctgacaatctcttccctggagcctgaggatttcgccgtgtactattgtcagcagagatctaattggccccctacctttggccagggcacaaaggtggagatcaagcgtacggtggccgctccttccgtgttcatctttccaccctctgacgagcagctgaagtctggcaccgcttccgtggtgtgcctgctgaacaacttctacccacgcgaggccaaggtgcagtggaaggtggataacgctctgcagtccggcaatagccaggagtctgtgacagagcaggactccaaggatagcacctattctctgtcttccaccctgacactgtctaaggccgattacgagaagcacaaggtgtatgcttgcgaggtgacacatcagggcctgagctctcccgtgaccaagtccttcaacagaggcgagtgt

SEQ ID NO: 10 - protein, 456 aa, Artificial Sequence
  Amino acid sequence of polypeptide chain H2 of MHI383-1122-IgG4
EVQLVESGGGLVQPGGSLRLSCAASGFTFNTYAMNWVRQAPGKGLEWVARIRSKYNNYATYYADSVKDRFTISRDDSKNTAYLQMNNLKTEDTAMYYCVRHGNFGNSYVSWFAYWGQGTLVTVSSGKETLQRADPPKTHVTHHPISRHEATLRCWALGFYPAEITLTWQRDGKDQTQKTELVETRPCGDRTFQKWAAVVVPSGEEQRYTCHVQHEGLPKPLTLRWEPSESKYGPPCPPCPAPEFLGGPSVFLFPPKPKDTLMISRTPEVTCVVVDVSQEDPEVQFNWYVDGVEVHNAKTKPREEQFNSTYRVVSVLTVLHQDWLNGKEYKCKVSNKGLPSSIEKTISKAKGQPREPQVCTLPPSQEEMTKNQVSLSCAVKGFYPSDIAVEWESNGQPENNYKTTPPVLDSDGSFFLVSRLTVDKSRWQEGNVFSCSVMHEALHNHYTQKSLSLSLG

SEQ ID NO: 11 - DNA, 1371 bp, Artificial Sequence
  Nucleotide sequence of polypeptide chain H2 of MHI383-1122-IgG4
gaggtgcagctggtggagtctggaggaggactggtgcagccaggaggaagcctgaggctgtcttgcgccgcttccggcttcacctttaacacatacgccatgaattgggtgagacaggctcctggcaagggactggagtgggtggctaggatccggtccaagtacaacaattatgccacctactatgctgacagcgtgaaggatagattcaccatcagccgcgacgattctaagaacacagcctatctgcagatgaacaatctgaagaccgaggacacagctatgtactattgcgtgaggcacggcaacttcggcaattcttacgtgtcctggtttgcttattggggccagggcaccctggtgacagtgtccagcggcaaggagaccctgcagagagctgacccccctaagacccacgtgacacaccatcccatctctagacatgaggccacactgaggtgctgggctctgggcttctaccctgccgagatcaccctgacatggcagcgcgacggcaaggatcagacccagaagacagagctggtggagaccaggccttgcggcgatcggacatttcagaagtgggctgctgtggtggtgccatccggagaggagcagaggtatacctgtcacgtgcagcatgagggcctgccaaagcccctgacactgcggtgggagccaagcgagagcaagtacggaccaccttgcccaccatgtccagctcctgagttcctgggaggaccatccgtgttcctgtttcctccaaagcccaaggacacactgatgatctctcggacaccagaggtgacctgcgtggtggtggacgtgtcccaggaggatcccgaggtgcagttcaactggtacgtggatggcgtggaggtgcacaatgccaagaccaagcccagagaggagcagtttaattccacataccgcgtggtgagcgtgctgaccgtgctgcatcaggattggctgaacggcaaggagtataagtgcaaggtgagcaataagggcctgccttccagcatcgagaagaccatctctaaggctaagggccagcctagggagccacaggtgtgcacactgccccctagccaggaggagatgaccaagaaccaggtgtccctgagctgtgccgtgaagggcttctaccccagcgacatcgctgtggagtgggagtctaatggccagcctgagaacaattataagaccacaccacccgtgctggacagcgatggctctttctttctggtgtctaggctgacagtggataagtcccggtggcaggagggcaacgtgttttcttgttccgtgatgcatgaggccctgcacaatcattacacccagaagagcctgtctctgtccctgggctga

SEQ ID NO: 12 - protein, 208 aa, Artificial Sequence
  Amino acid sequence of polypeptide chain L2 of MHI383-1122-IgG4
ELVVTQEPSLTTSPGGTVTLTCRSSTGAVTTSNYANWVQQKPGQAPRGLIGGTNKRAPGTPARFSGSLLGGKAALTITGVQPEDEAEYYCALWYSNLWVFGGGTKLTVLIQRTPKIQVYSCHPAENGKSNFLNCYVSGFHPSDIEVDLLKNGERIEKVEHSDLSFSKDWSFYLLYYTRFTPTEKDEYACRVNHVTLSQPKIVKWDRGP

SEQ ID NO: 13 - DNA, 624 bp, Artificial Sequence
  Nucleotide sequence of polypeptide chain L2 of MHI383-1122-IgG4
gagctggtggtgacacaggagcctagcctgaccacatctccaggcggcaccgtgacactgacctgcagatccagcaccggcgccgtgaccacatccaactacgctaattgggtgcagcagaagccaggacaggctccaaggggactgatcggaggaacaaacaagagggctccaggaacccctgctcggttctctggatccctgctgggaggcaaggccgctctgacaatcaccggagtgcagccagaggacgaggctgagtactattgtgctctgtggtatagcaatctgtgggtgtttggcggcggcacaaagctgaccgtgctgatccagagaacccccaagatccaggtgtacagctgccaccctgccgagaacggcaagtctaacttcctgaattgttacgtgtccggctttcatccttccgacatcgaggtggatctgctgaagaatggcgagcgcatcgagaaggtggagcactccgacctgtccttcagcaaggattggagcttttacctgctgtactataccaggttcaccccaacagagaaggacgagtatgcttgccgggtgaaccatgtgacactgtctcagccaaagatcgtgaagtgggataggggcccc

SEQ ID NO: 14 - protein, 452 aa, Artificial Sequence
  Amino acid sequence of polypeptide chain H3 of MHI383-1133-IgG4
EVQLVESGGGLVQPGGSLRLSCAASGFTFNTYAMNWVRQAPGKGLEWVARIRSKYNNYATYYADSVKDRFTISRDDSKNTAYLQMNNLKTEDTAMYYCVRHGNFGNSYVSWFAYWGQGTLVTVSSIQRTPKIQVYSCHPAENGKSNFLNCYVSGFHPSDIEVDLLKNGERIEKVEHSDLSFSKDWSFYLLYYTRFTPTEKDEYACRVNHVTLSQPKIVKWDRGPESKYGPPCPPCPAPEFLGGPSVFLFPPKPKDTLMISRTPEVTCVVVDVSQEDPEVQFNWYVDGVEVHNAKTKPREEQFNSTYRVVSVLTVLHQDWLNGKEYKCKVSNKGLPSSIEKTISKAKGQPREPQVCTLPPSQEEMTKNQVSLSCAVKGFYPSDIAVEWESNGQPENNYKTTPPVLDSDGSFFLVSRLTVDKSRWQEGNVFSCSVMHEALHNHYTQKSLSLSLG

SEQ ID NO: 15 - DNA, 1359 bp, Artificial Sequence
  Nucleotide sequence of polypeptide chain H3 of MHI383-1133-IgG4
gaggtgcagctggtggagtctggaggaggactggtgcagccaggaggaagcctgaggctgtcttgcgccgcttccggcttcacctttaacacatacgccatgaattgggtgagacaggctcctggcaagggactggagtgggtggctaggatccggtccaagtacaacaattatgccacctactatgctgacagcgtgaaggatagattcaccatcagccgcgacgattctaagaacacagcctatctgcagatgaacaatctgaagaccgaggacacagctatgtactattgcgtgaggcacggcaacttcggcaattcttacgtgtcctggtttgcttattggggccagggcaccctggtgacagtgtccagcatccagagaacccccaagatccaggtgtacagctgccaccctgccgagaacggcaagtctaacttcctgaattgttacgtgtccggctttcatccttccgacatcgaggtggatctgctgaagaatggcgagcgcatcgagaaggtggagcactccgacctgtccttcagcaaggattggagcttttacctgctgtactataccaggttcaccccaacagagaaggacgagtatgcttgccgggtgaaccatgtgacactgtctcagccaaagatcgtgaagtgggataggggccccgagagcaagtacggaccaccttgcccaccatgtccagctcctgagttcctgggaggaccatccgtgttcctgtttcctccaaagcccaaggacacactgatgatctctcggacaccagaggtgacctgcgtggtggtggacgtgtcccaggaggatcccgaggtgcagttcaactggtacgtggatggcgtggaggtgcacaatgccaagaccaagcccagagaggagcagtttaattccacataccgcgtggtgagcgtgctgaccgtgctgcatcaggattggctgaacggcaaggagtataagtgcaaggtgagcaataagggcctgccttccagcatcgagaagaccatctctaaggctaagggccagcctagggagccacaggtgtgcacactgccccctagccaggaggagatgaccaagaaccaggtgtccctgagctgtgccgtgaagggcttctaccccagcgacatcgctgtggagtgggagtctaatggccagcctgagaacaattataagaccacaccacccgtgctggacagcgatggctctttctttctggtgtctaggctgacagtggataagtcccggtggcaggagggcaacgtgttttcttgttccgtgatgcatgaggccctgcacaatcattacacccagaagagcctgtctctgtccctgggctga

SEQ ID NO: 16 - protein, 212 aa, Artificial Sequence
  Amino acid sequence of polypeptide chain L3 of MHI383-1133-IgG4
ELVVTQEPSLTTSPGGTVTLTCRSSTGAVTTSNYANWVQQKPGQAPRGLIGGTNKRAPGTPARFSGSLLGGKAALTITGVQPEDEAEYYCALWYSNLWVFGGGTKLTVLGKETLQRADPPKTHVTHHPISRHEATLRCWALGFYPAEITLTWQRDGKDQTQKTELVETRPCGDRTFQKWAAVVVPSGEEQRYTCHVQHEGLPKPLTLRWEPS

SEQ ID NO: 17 - DNA, 636 bp, Artificial Sequence
  Nucleotide sequence of polypeptide chain L3 of MHI383-1133-IgG4
gagctggtggtgacacaggagcctagcctgaccacatctccaggcggcaccgtgacactgacctgcagatccagcaccggcgccgtgaccacatccaactacgctaattgggtgcagcagaagccaggacaggctccaaggggactgatcggaggaacaaacaagagggctccaggaacccctgctcggttctctggatccctgctgggaggcaaggccgctctgacaatcaccggagtgcagccagaggacgaggctgagtactattgtgctctgtggtatagcaatctgtgggtgtttggcggcggcacaaagctgaccgtgctgggcaaggagaccctgcagagagctgacccccctaagacccacgtgacacaccatcccatctctagacatgaggccacactgaggtgctgggctctgggcttctaccctgccgagatcaccctgacatggcagcgcgacggcaaggatcagacccagaagacagagctggtggagaccaggccttgcggcgatcggacatttcagaagtgggctgctgtggtggtgccatccggagaggagcagaggtatacctgtcacgtgcagcatgagggcctgccaaagcccctgacactgcggtgggagccaagc

SEQ ID NO: 18 - protein, 452 aa, Artificial Sequence
  Amino acid sequence of Hc of MHI383-ccff-IgG1
EVQLLESGGGLVQPGGSLRLSCAVSGFTFNSFAMSWVRQAPGKGLEWVSAISGSGGGTYYADSVKGRFTISRDNSKNTLYLQMNSLRAEDTAVYFCAKDKILWFGEPVFDYWGQGTLVTVSSASTKGPSVFPLAPSSKSTSGGTAALGCLVKDYFPEPVTVSWNSGALTSGVHTFPAVLQSSGLYSLSSVVTVPSSSLGTQTYICNVNHKPSNTKVDKKVEPKSCDKTHTCPPCPAPEAAGGPSVFLFPPKPKDTLMISRTPEVTCVVVDVSHEDPEVKFNWYVDGVEVHNAKTKPREEQYNSTYRVVSVLTVLHQDWLNGKEYKCKVSNKALPAPIEKTISKAKGQPREPQVYTLPPCRDELTKNQVSLWCLVKGFYPSDIAVEWESNGQPENNYKTTPPVLDSDGSFFLYSKLTVDKSRWQQGNVFSCSVMHEALHNHYTQKSLSLSPGK

SEQ ID NO: 19 - DNA, 1356 bp, Artificial Sequence
  Nucleotide sequence of Hc of MHI383-ccff-IgG1
gaggtgcagctgctggagagcggaggaggactggtgcagccaggaggcagcctgagactgtcttgcgccgtgtccggcttcacctttaacagcttcgccatgtcttgggtgcgccaggctcctggcaagggactggagtgggtgtctgccatctctggatccggaggaggaacatactatgctgactccgtgaagggcaggttcaccatctcccgggataacagcaagaatacactgtacctgcagatgaattctctgagggccgaggacaccgccgtgtacttttgtgctaaggataagatcctgtggttcggcgagccagtgtttgactactggggccagggcaccctggtgacagtgtccagcgcctctaccaagggaccatccgtgttcccactggctccatccagcaagtccaccagcggaggaacagccgctctgggatgcctggtgaaggactacttcccagagcccgtgacagtgagctggaactctggcgccctgaccagcggagtgcacacatttccagctgtgctgcagtcttccggcctgtactctctgagctctgtggtgaccgtgccctccagctctctgggcacccagacatatatctgcaacgtgaatcacaagccaagcaatacaaaggtggacaagaaggtggagcccaagtcttgtgataagacccatacatgccccccttgtcctgctccagaggctgctggaggaccatccgtgttcctgtttccacccaagcctaaggacaccctgatgatctccaggacccccgaggtgacatgcgtggtggtggacgtgagccacgaggatcctgaggtgaagtttaactggtacgtggatggcgtggaggtgcataatgctaagaccaagcctagggaggagcagtacaacagcacctatcgggtggtgtctgtgctgacagtgctgcaccaggactggctgaacggcaaggagtataagtgtaaggtgtctaataaggccctgcccgctcctatcgagaagaccatctccaaggccaagggccagcctagagagccacaggtgtacaccctgcctccatgccgcgacgagctgacaaagaaccaggtgagcctgtggtgtctggtgaagggcttctatccttctgatatcgctgtggagtgggagtccaatggccagccagagaacaattacaagaccacaccccctgtgctggactccgatggcagcttctttctgtattccaagctgaccgtggataagagcagatggcagcagggcaacgtgttttcttgttccgtgatgcatgaggccctgcacaatcattatacacagaagagcctgtctctgtccccaggcaag

SEQ ID NO: 20 - protein, 214 aa, Artificial Sequence; identical to SEQ ID NO: 8
  Amino acid sequence of Lc of MHI383-ccff-IgG1

SEQ ID NO: 21 - DNA, 642 bp, Artificial Sequence; identical to SEQ ID NO: 9
  Nucleotide sequence of Lc of MHI383-ccff-IgG1

SEQ ID NO: 22 - protein, 460 aa, Artificial Sequence
  Amino acid sequence of Hf of MHI383-ccff-IgG1
EVQLVESGGGLVQPGGSLRLSCAASGFTFNTYAMNWVRQAPGKGLEWVARIRSKYNNYATYYADSVKDRFTISRDDSKNTAYLQMNNLKTEDTAMYYCVRHGNFGNSYVSWFAYWGQGTLVTVSSGKETLQRADPPKTHVTHHPISRHEATLRCWALGFYPAEITLTWQRDGKDQTQKTELVETRPCGDRTFQKWAAVVVPSGEEQRYTCHVQHEGLPKPLTLRWEPSEPKSSDKTHTCPPCPAPEAAGGPSVFLFPPKPKDTLMISRTPEVTCVVVDVSHEDPEVKFNWYVDGVEVHNAKTKPREEQYNSTYRVVSVLTVLHQDWLNGKEYKCKVSNKALPAPIEKTISKAKGQPREPQVCTLPPSRDELTKNQVSLSCAVKGFYPSDIAVEWESNGQPENNYKTTPPVLDSDGSFFLVSKLTVDKSRWQQGNVFSCSVMHEALHNRFTQKSLSLSPGK

SEQ ID NO: 23 - DNA, 1380 bp, Artificial Sequence
  Nucleotide sequence of Hf of MHI383-ccff-IgG1
gaggtgcagctggtggagtctggaggaggactggtgcagccaggaggaagcctgaggctgtcttgcgccgcttccggcttcacctttaacacatacgccatgaattgggtgagacaggctcctggcaagggactggagtgggtggctaggatccggtccaagtacaacaattatgccacctactatgctgacagcgtgaaggatagattcaccatcagccgcgacgattctaagaacacagcctatctgcagatgaacaatctgaagaccgaggacacagctatgtactattgcgtgaggcacggcaacttcggcaattcttacgtgtcctggtttgcttattggggccagggcaccctggtgacagtgtccagcggcaaggagaccctgcagagagctgacccccctaagacccacgtgacacaccatcccatctctagacatgaggccacactgaggtgctgggctctgggcttctaccctgccgagatcaccctgacatggcagcgcgacggcaaggatcagacccagaagacagagctggtggagaccaggccttgcggcgatcggacatttcagaagtgggctgctgtggtggtgccatccggagaggagcagaggtatacctgtcacgtgcagcatgagggcctgccaaagcccctgacactgcggtgggagccaagcgagccaaagtccagcgacaagacccacacatgcccaccttgtccagctccagaggctgctggaggaccatccgtgttcctgtttccacccaagcccaaggataccctgatgatctctaggacccccgaggtgacatgcgtggtggtggacgtgtcccacgaggatcctgaggtgaagttcaactggtacgtggacggcgtggaggtgcataatgccaagacaaagcccagggaggagcagtacaactctacctatcgggtggtgtccgtgctgacagtgctgcatcaggattggctgaacggcaaggagtataagtgtaaggtgagcaataaggccctgcctgctccaatcgagaagaccatctctaaggctaagggccagcccagagagcctcaggtgtgcaccctgcctccatcccgcgacgagctgacaaagaaccaggtgtctctgtcctgtgccgtgaagggcttttacccttccgatatcgctgtggagtgggagagcaatggccagccagagaacaattataagaccacaccccctgtgctggactccgatggcagcttctttctggtgagcaagctgaccgtggacaagtctaggtggcagcagggcaacgtgttcagctgctctgtgatgcacgaggctctgcataataggttcacccagaagtccctgagcctgtctcccggcaag

SEQ ID NO: 24 - protein, 208 aa, Artificial Sequence; identical to SEQ ID NO: 12
  Amino acid sequence of Lf of MHI383-ccff-IgG1

SEQ ID NO: 25 - DNA, 624 bp, Artificial Sequence; identical to SEQ ID NO: 13
  Nucleotide sequence of Lf of MHI383-ccff-IgG1

SEQ ID NO: 26 - protein, 446 aa, Artificial Sequence
  Amino acid sequence of heavy chain HZ5G11VH-CH1-IgG1
QITLKESGPTLVKPTQTLTLTCTVSGFSLSTYGVHWIRQPPGKALEWLGVIWRGVTTDYNAAFMSRLTITKDNSKNQVVLTMNNMDPVDTATYYCARLGFYAMDYWGQGTLVTVSSASTKGPSVFPLAPSSKSTSGGTAALGCLVKDYFPEPVTVSWNSGALTSGVHTFPAVLQSSGLYSLSSVVTVPSSSLGTQTYICNVNHKPSNTKVDKKVEPKSCDKTHTCPPCPAPELLGGPSVFLFPPKPKDTLMISRTPEVTCVVVDVSHEDPEVKFNWYVDGVEVHNAKTKPREEQYNSTYRVVSVLTVLHQDWLNGKEYKCKVSNKALPAPIEKTISKAKGQPREPQVYTLPPSRDELTKNQVSLTCLVKGFYPSDIAVEWESNGQPENNYKTTPPVLDSDGSFFLYSKLTVDKSRWQQGNVFSCSVMHEALHNHYTQKSLSLSPGK

SEQ ID NO: 27 - DNA, 1338 bp, Artificial Sequence
  Nucleotide sequence of heavy chain HZ5G11VH-CH1-IgG1
caaatcactctaaaggaaagtggtccaactctggtgaaacccacccagaccctgacactgacctgtaccgtgtctggctttagcctgtctacctacggcgtgcactggatcagacagcctcctggcaaggccctcgagtggctgggagtgatctggcggggcgtgaccaccgactataatgctgccttcatgtcccggctgaccatcaccaaggacaactccaagaaccaagtggtgctgaccatgaacaacatggatcctgtggacacagctacctactactgcgccagactgggcttctacgccatggactactggggccagggcaccctggtcacagtgtcctctgctagcacaaagggcccttccgtgttcccactggctccctcttccaagtctacatccggaggaaccgccgctctgggatgcctggtgaaggattatttcccagagcccgtgaccgtgtcttggaactccggcgccctgacaagcggagtgcatacctttcctgctgtgctgcagagctctggcctgtattctctgtccagcgtggtgacagtgccatcttccagcctgggcacccagacatacatctgcaacgtgaatcacaagcctagcaataccaaggtggacaagaaggtggagccaaagtcttgtgataagacccatacatgccccccttgtcctgctccagagctgctgggaggaccatccgtgttcctgtttccacccaagcccaaggacaccctgatgatctcccgcacaccagaggtgacctgcgtggtggtggacgtgagccacgaggatcccgaggtgaagtttaactggtacgtggatggcgtggaggtgcataatgctaagaccaagccaagagaggagcagtataacagcacataccgcgtggtgtctgtgctgaccgtgctgcaccaggactggctgaacggcaaggagtacaagtgcaaggtgtctaataaggccctgcccgctcctatcgagaagacaatctccaaggccaagggccagcctagggagccacaggtgtataccctgcctccatctcgggacgagctgacaaagaaccaggtgtccctgacctgtctggtgaagggcttctaccccagcgatatcgctgtggagtgggagtctaatggccagcctgagaacaattataagaccacaccccctgtgctggacagcgatggctctttctttctgtactctaagctgacagtggataagtccaggtggcagcagggcaacgtgtttagctgctctgtgatgcatgaggctctgcacaatcattacacccagaagtccctgagcctgtctcccggcaag

SEQ ID NO: 28 - protein, 214 aa, Artificial Sequence
  Amino acid sequence of light chain HZ5G11VL-IgK
DIQMTQSPSSLSASVGDRVTITCKASQSVSNDVAWYQQKPGKAPKLLIYYAANRYTGVPDRFSGSGYGTDFTFTISSLQPEDIATYFCQQDYTSPYTFGQGTKLEIKRTVAAPSVFIFPPSDEQLKSGTASVVCLLNNFYPREAKVQWKVDNALQSGNSQESVTEQDSKDSTYSLSSTLTLSKADYEKHKVYACEVTHQGLSSPVTKSFNRGEC

SEQ ID NO: 29 - DNA, 642 bp, Artificial Sequence
  Nucleotide sequence of light chain HZ5G11VL-IgK
gatatccaaatgactcaaagtccaagtagtctgtccgcttctgtcggcgacagagtgaccatcacctgtaaggcctctcagtccgtgtccaacgacgtggcttggtaccagcagaagcctggcaaggctcctaagctgctgatctactacgccgccaaccggtacaccggcgtgcccgatagattctccggctctggctacggcaccgacttcacctttacaatctccagcctgcagcctgaggatatcgccacctacttctgccagcaggactacacctctccatataccttcggccaaggaacaaaactggaaatcaagcgtacggtggccgctccttccgtgttcatctttcccccttccgatgagcagctgaagagcggcacagcttctgtggtgtgcctgctgaacaacttctacccaagggaggccaaggtgcagtggaaggtggacaacgctctgcagagcggcaattctcaggagtccgtgaccgagcaggacagcaaggattctacatattccctgtccagcaccctgacactgtccaaggccgattacgagaagcacaaggtgtatgcttgcgaggtgacccatcagggcctgtcttcccccgtgacaaagagctttaatagaggcgagtgt

SEQ ID NO: 30 - protein, 451 aa, Artificial Sequence
  Amino acid sequence of heavy chain HZ5G11VH-Cα-IgG1
QITLKESGPTLVKPTQTLTLTCTVSGFSLSTYGVHWIRQPPGKALEWLGVIWRGVTTDYNAAFMSRLTITKDNSKNQVVLTMNNMDPVDTATYYCARLGFYAMDYWGQGTLVTVSSGKETLQRADPPKTHVTHHPISRHEATLRCWALGFYPAEITLTWQRDGKDQTQKTELVETRPCGDRTFQKWAAVVVPSGEEQRYTCHVQHEGLPKPLTLRWEPSEPKSCDKTHTCPPCPAPELLGGPSVFLFPPKPKDTLMISRTPEVTCVVVDVSHEDPEVKFNWYVDGVEVHNAKTKPREEQYNSTYRVVSVLTVLHQDWLNGKEYKCKVSNKALPAPIEKTISKAKGQPREPQVYTLPPSRDELTKNQVSLTCLVKGFYPSDIAVEWESNGQPENNYKTTPPVLDSDGSFFLYSKLTVDKSRWQQGNVFSCSVMHEALHNHYTQKSLSLSPGK

SEQ ID NO: 31 - DNA, 1353 bp, Artificial Sequence
  Nucleotide sequence of heavy chain HZ5G11VH-Cα-IgG1
caaatcactctaaaggaaagtggtccaactctggtgaaacccacccagaccctgacactgacctgtaccgtgtctggctttagcctgtctacctacggcgtgcactggatcagacagcctcctggcaaggccctcgagtggctgggagtgatctggcggggcgtgaccaccgactataatgctgccttcatgtcccggctgaccatcaccaaggacaactccaagaaccaagtggtgctgaccatgaacaacatggatcctgtggacacagctacctactactgcgccagactgggcttctacgccatggactactggggccagggcaccctggtcacagtgtcctctggcaaggagaccctgcagagagctgacccccctaagacccacgtgacacaccatcccatctctagacatgaggccacactgaggtgctgggctctgggcttctaccctgccgagatcaccctgacatggcagcgcgacggcaaggatcagacccagaagacagagctggtggagaccaggccttgcggcgatcggacatttcagaagtgggctgctgtggtggtgccatccggagaggagcagaggtatacctgtcacgtgcagcatgagggcctgccaaagcccctgacactgcggtgggagccaagcgagccaaagtcttgtgataagacccatacatgccccccttgtcctgctccagagctgctgggaggaccatccgtgttcctgtttccacccaagcccaaggacaccctgatgatctcccgcacaccagaggtgacctgcgtggtggtggacgtgagccacgaggatcccgaggtgaagtttaactggtacgtggatggcgtggaggtgcataatgctaagaccaagccaagagaggagcagtataacagcacataccgcgtggtgtctgtgctgaccgtgctgcaccaggactggctgaacggcaaggagtacaagtgcaaggtgtctaataaggccctgcccgctcctatcgagaagacaatctccaaggccaagggccagcctagggagccacaggtgtataccctgcctccatctcgggacgagctgacaaagaaccaggtgtccctgacctgtctggtgaagggcttctaccccagcgatatcgctgtggagtgggagtctaatggccagcctgagaacaattataagaccacaccccctgtgctggacagcgatggctctttctttctgtactctaagctgacagtggataagtccaggtggcagcagggcaacgtgtttagctgctctgtgatgcatgaggctctgcacaatcattacacccagaagtccctgagcctgtctcccggcaag

SEQ ID NO: 32 - protein, 206 aa, Artificial Sequence
  Amino acid sequence of light chain HZ5G11VL-Cβ
DIQMTQSPSSLSASVGDRVTITCKASQSVSNDVAWYQQKPGKAPKLLIYYAANRYTGVPDRFSGSGYGTDFTFTISSLQPEDIATYFCQQDYTSPYTFGQGTKLEIKIQRTPKIQVYSCHPAENGKSNFLNCYVSGFHPSDIEVDLLKNGERIEKVEHSDLSFSKDWSFYLLYYTRFTPTEKDEYACRVNHVTLSQPKIVKWDRGP

SEQ ID NO: 33 - DNA, 618 bp, Artificial Sequence
  Nucleotide sequence of light chain HZ5G11VL-Cβ
gatatccaaatgactcaaagtccaagtagtctgtccgcttctgtcggcgacagagtgaccatcacctgtaaggcctctcagtccgtgtccaacgacgtggcttggtaccagcagaagcctggcaaggctcctaagctgctgatctactacgccgccaaccggtacaccggcgtgcccgatagattctccggctctggctacggcaccgacttcacctttacaatctccagcctgcagcctgaggatatcgccacctacttctgccagcaggactacacctctccatataccttcggccaaggaacaaaactggaaatcaagatccagagaacccccaagatccaggtgtacagctgccaccctgccgagaacggcaagtctaacttcctgaattgttacgtgtccggctttcatccttccgacatcgaggtggatctgctgaagaatggcgagcgcatcgagaaggtggagcactccgacctgtccttcagcaaggattggagcttttacctgctgtactataccaggttcaccccaacagagaaggacgagtatgcttgccgggtgaaccatgtgacactgtctcagccaaagatcgtgaagtgggataggggcccc

SEQ ID NO: 34 - protein, 98 aa, Artificial Sequence
  Wild type amino acid sequence of constant region CH1 of IgG1
ASTKGPSVFPLAPSSKSTSGGTAALGCLVKDYFPEPVTVSWNSGALTSGVHTFPAVLQSSGLYSLSSVVTVPSSSLGTQTYICNVNHKPSNTKVDKKV

SEQ ID NO: 35 - protein, 107 aa, Artificial Sequence [sequence omitted]

SEQ ID NO: 36 - protein, 214 aa, Artificial Sequence
  Amino acid sequence of HZ5G11VL-IgK-S114A
DIQMTQSPSSLSASVGDRVTITCKASQSVSNDVAWYQQKPGKAPKLLIYYAANRYTGVPDRFSGSGYGTDFTFTISSLQPEDIATYFCQQDYTSPYTFGQGTKLEIKRTVAAPAVFIFPPSDEQLKSGTASVVCLLNNFYPREAKVQWKVDNALQSGNSQESVTEQDSKDSTYSLSSTLTLSKADYEKHKVYACEVTHQGLSSPVTKSFNRGEC

SEQ ID NO: 37 - DNA, 642 bp, Artificial Sequence
  Nucleotide sequence of HZ5G11VL-IgK-S114A
gatatccaaatgactcaaagtccaagtagtctgtccgcttctgtcggcgacagagtgaccatcacctgtaaggcctctcagtccgtgtccaacgacgtggcttggtaccagcagaagcctggcaaggctcctaagctgctgatctactacgccgccaaccggtacaccggcgtgcccgatagattctccggctctggctacggcaccgacttcacctttacaatctccagcctgcagcctgaggatatcgccacctacttctgccagcaggactacacctctccatataccttcggccaaggaacaaaactggaaatcaagcgtacggtggccgctcctgccgtgttcatctttcccccttccgatgagcagctgaagagcggcacagcttctgtggtgtgcctgctgaacaacttctacccaagggaggccaaggtgcagtggaaggtggacaacgctctgcagagcggcaattctcaggagtccgtgaccgagcaggacagcaaggattctacatattccctgtccagcaccctgacactgtccaaggccgattacgagaagcacaaggtgtatgcttgcgaggtgacccatcagggcctgtcttcccccgtgacaaagagctttaatagaggcgagtgt

SEQ ID NO: 38 - protein, 214 aa, Artificial Sequence
  Amino acid sequence of HZ5G11VL-IgK-F116A
DIQMTQSPSSLSASVGDRVTITCKASQSVSNDVAWYQQKPGKAPKLLIYYAANRYTGVPDRFSGSGYGTDFTFTISSLQPEDIATYFCQQDYTSPYTFGQGTKLEIKRTVAAPSVAIFPPSDEQLKSGTASVVCLLNNFYPREAKVQWKVDNALQSGNSQESVTEQDSKDSTYSLSSTLTLSKADYEKHKVYACEVTHQGLSSPVTKSFNRGEC

SEQ ID NO: 39 - DNA, 642 bp, Artificial Sequence
  Nucleotide sequence of HZ5G11VL-IgK-F116A
gatatccaaatgactcaaagtccaagtagtctgtccgcttctgtcggcgacagagtgaccatcacctgtaaggcctctcagtccgtgtccaacgacgtggcttggtaccagcagaagcctggcaaggctcctaagctgctgatctactacgccgccaaccggtacaccggcgtgcccgatagattctccggctctggctacggcaccgacttcacctttacaatctccagcctgcagcctgaggatatcgccacctacttctgccagcaggactacacctctccatataccttcggccaaggaacaaaactggaaatcaagcgtacggtggccgctccttccgtggccatctttcccccttccgatgagcagctgaagagcggcacagcttctgtggtgtgcctgctgaacaacttctacccaagggaggccaaggtgcagtggaaggtggacaacgctctgcagagcggcaattctcaggagtccgtgaccgagcaggacagcaaggattctacatattccctgtccagcaccctgacactgtccaaggccgattacgagaagcacaaggtgtatgcttgcgaggtgacccatcagggcctgtcttcccccgtgacaaagagctttaatagaggcgagtgt

SEQ ID NO: 40 - protein, 214 aa, Artificial Sequence
  Amino acid sequence of HZ5G11VL-IgK-F118A
DIQMTQSPSSLSASVGDRVTITCKASQSVSNDVAWYQQKPGKAPKLLIYYAANRYTGVPDRFSGSGYGTDFTFTISSLQPEDIATYFCQQDYTSPYTFGQGTKLEIKRTVAAPSVFIAPPSDEQLKSGTASVVCLLNNFYPREAKVQWKVDNALQSGNSQESVTEQDSKDSTYSLSSTLTLSKADYEKHKVYACEVTHQGLSSPVTKSFNRGEC

SEQ ID NO: 41 - DNA, 642 bp, Artificial Sequence
  Nucleotide sequence of HZ5G11VL-IgK-F118A
gatatccaaatgactcaaagtccaagtagtctgtccgcttctgtcggcgacagagtgaccatcacctgtaaggcctctcagtccgtgtccaacgacgtggcttggtaccagcagaagcctggcaaggctcctaagctgctgatctactacgccgccaaccggtacaccggcgtgcccgatagattctccggctctggctacggcaccgacttcacctttacaatctccagcctgcagcctgaggatatcgccacctacttctgccagcaggactacacctctccatataccttcggccaaggaacaaaactggaaatcaagcgtacggtggccgctccttccgtgttcatcgctcccccttccgatgagcagctgaagagcggcacagcttctgtggtgtgcctgctgaacaacttctacccaagggaggccaaggtgcagtggaaggtggacaacgctctgcagagcggcaattctcaggagtccgtgaccgagcaggacagcaaggattctacatattccctgtccagcaccctgacactgtccaaggccgattacgagaagcacaaggtgtatgcttgcgaggtgacccatcagggcctgtcttcccccgtgacaaagagctttaatagaggcgagtgt

SEQ ID NO: 42 - protein, 214 aa, Artificial Sequence
  Amino acid sequence of HZ5G11VL-IgK-F118I
DIQMTQSPSSLSASVGDRVTITCKASQSVSNDVAWYQQKPGKAPKLLIYYAANRYTGVPDRFSGSGYGTDFTFTISSLQPEDIATYFCQQDYTSPYTFGQGTKLEIKRTVAAPSVFIIPPSDEQLKSGTASVVCLLNNFYPREAKVQWKVDNALQSGNSQESVTEQDSKDSTYSLSSTLTLSKADYEKHKVYACEVTHQGLSSPVTKSFNRGEC

SEQ ID NO: 43 - DNA, 642 bp, Artificial Sequence
  Nucleotide sequence of HZ5G11VL-IgK-F118I
gatatccaaatgactcaaagtccaagtagtctgtccgcttctgtcggcgacagagtgaccatcacctgtaaggcctctcagtccgtgtccaacgacgtggcttggtaccagcagaagcctggcaaggctcctaagctgctgatctactacgccgccaaccggtacaccggcgtgcccgatagattctccggctctggctacggcaccgacttcacctttacaatctccagcctgcagcctgaggatatcgccacctacttctgccagcaggactacacctctccatataccttcggccaaggaacaaaactggaaatcaagcgtacggtggccgctccttccgtgttcatcattcccccttccgatgagcagctgaagagcggcacagcttctgtggtgtgcctgctgaacaacttctacccaagggaggccaaggtgcagtggaaggtggacaacgctctgcagagcggcaattctcaggagtccgtgaccgagcaggacagcaaggattctacatattccctgtccagcaccctgacactgtccaaggccgattacgagaagcacaaggtgtatgcttgcgaggtgacccatcagggcctgtcttcccccgtgacaaagagctttaatagaggcgagtgt

SEQ ID NO: 44 - protein, 107 aa, Artificial Sequence
  Amino acid sequence of CL domain containing F118A
RTVAAPSVFIAPPSDEQLKSGTASVVCLLNNFYPREAKVQWKVDNALQSGNSQESVTEQDSKDSTYSLSSTLTLSKADYEKHKVYACEVTHQGLSSPVTKSFNRGEC

SEQ ID NO: 45 - protein, 450 aa, Artificial Sequence
  Amino acid sequence of HZ14A9VH-CH1-IgG1
QVQLVQSGAEVKKPGASVKVSCKVSGFNIEDDYIEWVRQAPGQGLEWMGRIDPANDKTKYAQKFQGRVTMTGDTSTNTVYMELSSLRSEDTAVYYCARPGLRRYYSMDYWGQGTLVTVSSASTKGPSVFPLAPSSKSTSGGTAALGCLVKDYFPEPVTVSWNSGALTSGVHTFPAVLQSSGLYSLSSVVTVPSSSLGTQTYICNVNHKPSNTKVDKKVEPKSCDKTHTCPPCPAPELLGGPSVFLFPPKPKDTLMISRTPEVTCVVVDVSHEDPEVKFNWYVDGVEVHNAKTKPREEQYNSTYRVVSVLTVLHQDWLNGKEYKCKVSNKALPAPIEKTISKAKGQPREPQVYTLPPSRDELTKNQVSLTCLVKGFYPSDIAVEWESNGQPENNYKTTPPVLDSDGSFFLYSKLTVDKSRWQQGNVFSCSVMHEALHNHYTQKSLSLSPGK

SEQ ID NO: 46 - protein, 214 aa, Artificial Sequence
  Amino acid sequence of HZ14A9VL-IgK
DIQMTQSPSSLSASVGDRVTITCKASENVVSYVSWYQQKPGKAPKLLIYGASNRYTGVPSRFIGSGSSTDFTLTISSLQPEDFATYYCGQSYSYPLTFGQGTKLEIKRTVAAPSVFIFPPSDEQLKSGTASVVCLLNNFYPREAKVQWKVDNALQSGNSQESVTEQDSKDSTYSLSSTLTLSKADYEKHKVYACEVTHQGLSSPVTKSFNRGEC

SEQ ID NO: 47 - protein, 455 aa, Artificial Sequence
  Amino acid sequence of HZ14A9VH-Cα-IgG1
QVQLVQSGAEVKKPGASVKVSCKVSGFNIEDDYIEWVRQAPGQGLEWMGRIDPANDKTKYAQKFQGRVTMTGDTSTNTVYMELSSLRSEDTAVYYCARPGLRRYYSMDYWGQGTLVTVSSGKETLQRADPPKTHVTHHPISRHEATLRCWALGFYPAEITLTWQRDGKDQTQKTELVETRPCGDRTFQKWAAVVVPSGEEQRYTCHVQHEGLPKPLTLRWEPSEPKSCDKTHTCPPCPAPELLGGPSVFLFPPKPKDTLMISRTPEVTCVVVDVSHEDPEVKFNWYVDGVEVHNAKTKPREEQYNSTYRVVSVLTVLHQDWLNGKEYKCKVSNKALPAPIEKTISKAKGQPREPQVYTLPPSRDELTKNQVSLTCLVKGFYPSDIAVEWESNGQPENNYKTTPPVLDSDGSFFLYSKLTVDKSRWQQGNVFSCSVMHEALHNHYTQKSLSLSPGK

SEQ ID NO: 48 - protein, 206 aa, Artificial Sequence
  Amino acid sequence of HZ14A9VL-Cβ
DIQMTQSPSSLSASVGDRVTITCKASENVVSYVSWYQQKPGKAPKLLIYGASNRYTGVPSRFIGSGSSTDFTLTISSLQPEDFATYYCGQSYSYPLTFGQGTKLEIKIQRTPKIQVYSCHPAENGKSNFLNCYVSGFHPSDIEVDLLKNGERIEKVEHSDLSFSKDWSFYLLYYTRFTPTEKDEYACRVNHVTLSQPKIVKWDRGP

SEQ ID NO: 49 - protein, 451 aa, Artificial Sequence
  Amino acid sequence of H2 of MHL147-3322-IgG1-wt/MHL147-3322-F118A
QITLKESGPTLVKPTQTLTLTCTVSGFSLSTYGVHWIRQPPGKALEWLGVIWRGVTTDYNAAFMSRLTITKDNSKNQVVLTMNNMDPVDTATYYCARLGFYAMDYWGQGTLVTVSSGKETLQRADPPKTHVTHHPISRHEATLRCWALGFYPAEITLTWQRDGKDQTQKTELVETRPCGDRTFQKWAAVVVPSGEEQRYTCHVQHEGLPKPLTLRWEPSEPKSSDKTHTCPPCPAPEAAGGPSVFLFPPKPKDTLMISRTPEVTCVVVDVSHEDPEVKFNWYVDGVEVHNAKTKPREEQYNSTYRVVSVLTVLHQDWLNGKEYKCKVSNKALPAPIEKTISKAKGQPREPQVCTLPPSRDELTKNQVSLSCAVKGFYPSDIAVEWESNGQPENNYKTTPPVLDSDGSFFLVSKLTVDKSRWQQGNVFSCSVMHEALHNRFTQKSLSLSPGK

SEQ ID NO: 50 - protein, 206 aa, Artificial Sequence; identical to SEQ ID NO: 32
  Amino acid sequence of L2 of MHL147-3322-IgG1-wt/MHL147-3322-F118A

SEQ ID NO: 51 - protein, 450 aa, Artificial Sequence
  Amino acid sequence of H3 of MHL147-3322-IgG1-wt/MHL147-3322-F118A
QVQLVQSGAEVKKPGASVKVSCKVSGFNIEDDYIEWVRQAPGQGLEWMGRIDPANDKTKYAQKFQGRVTMTGDTSTNTVYMELSSLRSEDTAVYYCARPGLRRYYSMDYWGQGTLVTVSSASTKGPSVFPLAPSSKSTSGGTAALGCLVKDYFPEPVTVSWNSGALTSGVHTFPAVLQSSGLYSLSSVVTVPSSSLGTQTYICNVNHKPSNTKVDKKVEPKSCDKTHTCPPCPAPEAAGGPSVFLFPPKPKDTLMISRTPEVTCVVVDVSHEDPEVKFNWYVDGVEVHNAKTKPREEQYNSTYRVVSVLTVLHQDWLNGKEYKCKVSNKALPAPIEKTISKAKGQPREPQVYTLPPCRDELTKNQVSLWCLVKGFYPSDIAVEWESNGQPENNYKTTPPVLDSDGSFFLYSKLTVDKSRWQQGNVFSCSVMHEALHNHYTQKSLSLSPGK

SEQ ID NO: 52 - protein, 214 aa, Artificial Sequence
  Amino acid sequence of L3 of MHL147-3322-F118A
DIQMTQSPSSLSASVGDRVTITCKASENVVSYVSWYQQKPGKAPKLLIYGASNRYTGVPSRFIGSGSSTDFTLTISSLQPEDFATYYCGQSYSYPLTFGQGTKLEIKRTVAAPSVFIAPPSDEQLKSGTASVVCLLNNFYPREAKVQWKVDNALQSGNSQESVTEQDSKDSTYSLSSTLTLSKADYEKHKVYACEVTHQGLSSPVTKSFNRGEC

SEQ ID NO: 53 - protein, 214 aa, Artificial Sequence; identical to SEQ ID NO: 46
  Amino acid sequence of L3 of MHL147-3322-IgG1-wt